European Patent Specification EP 4 077 717 B1, published February 28, 2024. Title: METHOD OF DETECTING AN ANALYTE. Applicant: CartaNA AB 10x Genomics, Inc. Application Not Yet Assigned. The sequence listing filed with the application follows.

SEQUENCE LISTING (49 sequences)

SEQ ID NO: 1 - DNA, 25 bp, Artificial Sequence
  Synthetic construct
cctctattgttggatcatattcgtc

SEQ ID NO: 2 - DNA, 20 bp, Artificial Sequence
  Synthetic construct
cgggcggcggatcggcaaag

SEQ ID NO: 3 - DNA, 73 bp, Artificial Sequence
  Synthetic construct
tggcgtaggcaagagagtagccgtgactatcgactcctcaatgctgctgctgtactacggtagttggagctgg

SEQ ID NO: 4 - DNA, 73 bp, Artificial Sequence
  Synthetic construct
tggcgtaggcaagagcctcaatgcacatgtttggctccagtcggaagtactactctctggtagttggagctga

SEQ ID NO: 5 - DNA, 84 bp, Artificial Sequence
  Synthetic construct
agcctcgcctttgcctcctctatgattactgactgcgtctatttagtggagccacgactatcttctttcgccccgcgagcacag

SEQ ID NO: 6 - DNA, 23 bp, Artificial Sequence
  Synthetic construct
cctcaatgctgctgctgtactac

SEQ ID NO: 7 - DNA, 20 bp, Artificial Sequence
  Synthetic construct
agtcggaagtactactctct

SEQ ID NO: 8 - DNA, 20 bp, Artificial Sequence
  Synthetic construct
tgcgtctatttagtggagcc

SEQ ID NO: 9 - DNA, 41 bp, Artificial Sequence
  Synthetic construct
agctcagtccatcctcgtaatcaatgctgctgctgtactac

SEQ ID NO: 10 - DNA, 40 bp, Artificial Sequence
  Synthetic construct
agtagccgtgactatcgactaaaaatcctcatcaatcatc

SEQ ID NO: 11 - DNA, 40 bp, Artificial Sequence
  Synthetic construct
cacatttacagacctcaaatagtcggaagtactactctct

SEQ ID NO: 12 - DNA, 41 bp, Artificial Sequence
  Synthetic construct
cctcaatgcacatgtttggctatcctacctccaactctcac

SEQ ID NO: 13 - DNA, 40 bp, Artificial Sequence
  Synthetic construct
ctcactcccaatctctataaggcgtaggcaagagtcctag

SEQ ID NO: 14 - DNA, 40 bp, Artificial Sequence
  Synthetic construct
tcaaagggtagttggagctgaactaccctacaaatccaat

SEQ ID NO: 15 - DNA, 45 bp, Artificial Sequence
  Synthetic construct
gtccctgcctctatatcttttgcctcctctatgattactgactgc

SEQ ID NO: 16 - DNA, 45 bp, Artificial Sequence
  Synthetic construct
cgccccgcgagcacagagcctcgccttccactcaactttaacccg

SEQ ID NO: 17 - DNA, 91 bp, Artificial Sequence
  Synthetic construct
gttttctttcagacagaatctgcgtctatttagtggagccactgctatctacgtagctagacgttgtcttagttggtattattgtcatttt

SEQ ID NO: 18 - DNA, 80 bp, Artificial Sequence
  Synthetic construct
agcaacgcaaacctgtctgcgtctatttagtggagccacacctatctagctagctactcgttgtccaccatcacggaccg

SEQ ID NO: 19 - DNA, 81 bp, Artificial Sequence
  Synthetic construct
agctcccgtgccaactgcgtctatttagtggagcccacactatctatatagctacgagttgtcatgaattatgccgacatc

SEQ ID NO: 20 - DNA, 82 bp, Artificial Sequence
  Synthetic construct
ataccctcaccatcttctgcgtctatttagtggagccgaaactatctcagtagctacctgttgtctcattgtgtaggagtgc

SEQ ID NO: 21 - DNA, 83 bp, Artificial Sequence
  Synthetic construct
tgtcccttctacaagcatgcgtctatttagtggagccggccctatctccttagctacaggttgtcgttctcattttctaccac

SEQ ID NO: 22 - DNA, 83 bp, Artificial Sequence
  Synthetic construct
cctacaccaacaatgagatgcgtctatttagtggagcccaacctatctcgatagctaatagttgtccgtccacaaccacaaca

SEQ ID NO: 23 - DNA, 82 bp, Artificial Sequence
  Synthetic construct
gggcagaagaaagtcctgcgtctatttagtggagccaagactatctctctagctaagcgttgtcacgtcaggagataatgat

SEQ ID NO: 24 - DNA, 81 bp, Artificial Sequence
  Synthetic construct
cctggattcttcttggtgcgtctatttagtggagcctggtctatctgactagctaacggttgtctgtcattgctgaggtag

SEQ ID NO: 25 - DNA, 61 bp, Artificial Sequence
  Synthetic construct
ctcactcccaatctctatctaccctacaaatccaataaaaatgcgtctatttagtggagcc

SEQ ID NO: 26 - DNA, 55 bp, Artificial Sequence
  Synthetic construct
tagctagacgttgttaaaaaaagtctaatccgtccctgcctctatatctccactc

SEQ ID NO: 27 - DNA, 55 bp, Artificial Sequence
  Synthetic construct
tagctactcgttgttaaaaaaagtctaatccgtccctgcctctatatctccactc

SEQ ID NO: 28 - DNA, 55 bp, Artificial Sequence
  Synthetic construct
tagctacgagttgtattttcacatttacagacctcaacctacctccaactctcac

SEQ ID NO: 29 - DNA, 55 bp, Artificial Sequence
  Synthetic construct
tagctacctgttgttaaaaaaagtctaatccgtccctgcctctatatctccactc

SEQ ID NO: 30 - DNA, 55 bp, Artificial Sequence
  Synthetic construct
tagctacaggttgttaaaaaaagtctaatccgtccctgcctctatatctccactc

SEQ ID NO: 31 - DNA, 55 bp, Artificial Sequence
  Synthetic construct
tagctaatagttgtattttcacatttacagacctcaacctacctccaactctcac

SEQ ID NO: 32 - DNA, 55 bp, Artificial Sequence
  Synthetic construct
tagctaagcgttgtattttcacatttacagacctcaacctacctccaactctcac

SEQ ID NO: 33 - DNA, 55 bp, Artificial Sequence
  Synthetic construct
tagctaacggttgtattttcacatttacagacctcaacctacctccaactctcac

SEQ ID NO: 34 - DNA, 55 bp, Artificial Sequence
  Synthetic construct
tagctagacgttgtatatagcattctttcttgaggagggcagcaaacgggaagag

SEQ ID NO: 35 - DNA, 55 bp, Artificial Sequence; identical to SEQ ID NO: 27
  Synthetic construct

SEQ ID NO: 36 - DNA, 55 bp, Artificial Sequence
  Synthetic construct
tagctacgagttgtatatagcattctttcttgaggagggcagcaaacgggaagag

SEQ ID NO: 37 - DNA, 55 bp, Artificial Sequence
  Synthetic construct
tagctacctgttgtattttcacatttacagacctcaacctacctccaactctcac

SEQ ID NO: 38 - DNA, 55 bp, Artificial Sequence
  Synthetic construct
tagctacaggttgtaaaaaagctcagtccatcctcgtaaatcctcatcaatcatc

SEQ ID NO: 39 - DNA, 55 bp, Artificial Sequence; identical to SEQ ID NO: 31
  Synthetic construct

SEQ ID NO: 40 - DNA, 55 bp, Artificial Sequence
  Synthetic construct
tagctaagcgttgttaaaaaaagtctaatccgtccctgcctctatatctccactc

SEQ ID NO: 41 - DNA, 55 bp, Artificial Sequence
  Synthetic construct
tagctaacggttgtaaaaaagctcagtccatcctcgtaaatcctcatcaatcatc

SEQ ID NO: 42 - DNA, 55 bp, Artificial Sequence; identical to SEQ ID NO: 26
  Synthetic construct

SEQ ID NO: 43 - DNA, 55 bp, Artificial Sequence
  Synthetic construct
tagctactcgttgtatatagcattctttcttgaggagggcagcaaacgggaagag

SEQ ID NO: 44 - DNA, 55 bp, Artificial Sequence; identical to SEQ ID NO: 28
  Synthetic construct

SEQ ID NO: 45 - DNA, 55 bp, Artificial Sequence
  Synthetic construct
tagctacctgttgtaaaaaagctcagtccatcctcgtaaatcctcatcaatcatc

SEQ ID NO: 46 - DNA, 55 bp, Artificial Sequence
  Synthetic construct
tagctacaggttgtattttcacatttacagacctcaacctacctccaactctcac

SEQ ID NO: 47 - DNA, 55 bp, Artificial Sequence
  Synthetic construct
tagctaatagttgtatatagcattctttcttgaggagggcagcaaacgggaagag

SEQ ID NO: 48 - DNA, 55 bp, Artificial Sequence
  Synthetic construct
tagctaagcgttgtaaaaaagctcagtccatcctcgtaaatcctcatcaatcatc

SEQ ID NO: 49 - DNA, 55 bp, Artificial Sequence
  Synthetic construct
tagctaacggttgttaaaaaaagtctaatccgtccctgcctctatatctccactc